European Patent Application EP 4 382 609 A1, published June 12, 2024. Title: Fusion protein of antigen-binding molecule and streptavidin mutant. Applicant: Savid Therapeutics Inc. The sequence listing filed with the application follows.

SEQUENCE LISTING (18 sequences)

SEQ ID NO: 1 - protein, 133 aa, synthetic construct
  REGION 1..133: note = Description of Artificial Sequence: Recombinant protein
AEAGITGTWSNQLGSTFIVTAGADGALTGTYESAVGNAESRYVLTGRYDSAPATDGSGTALGWTVAWKNNSKNAHSATTWSGQYVGGADAKINTQWLLTSGTTNANAWKSTLVGHDTFTKVKPSAASHHHHHH

SEQ ID NO: 2 - skipped

SEQ ID NO: 3 - protein, 211 aa, synthetic construct
  REGION 1..211: note = Description of Artificial Sequence: Recombinant protein
MVDNKFNKEMRNAYWEIALLPNLNNQQKRAFIRSIYDDPSQSANLLAEAKKLNDAQAPKSGGGGGSGGGGGSGGGGGSAEAGITGTWSNQLGSTFIVTAGADGALTGTYESAVGNAESRYVLTGRYDSAPATDGSGTALGWTVAWKNNSKNAHSATTWSGQYVGGADAKINTQWLLTSGTTNANAWKSTLVGHDTFTKVKPSAASHHHHHH

SEQ ID NO: 4 - DNA, 636 bp, synthetic construct
  misc_feature 1..636: note = Description of Artificial Sequence: Recombinant DNA
  source 1..636: mol_type = other DNA
atggtggacaacaaattcaacaaagagatgcgcaatgcgtactgggaaattgccctgttaccgaacctgaacaaccagcagaaacgtgccttcattcgcagcatctatgacgatccaagccaatctgcgaatctgcttgcagaagcgaagaaactgaatgatgctcaagctccgaaaagcggaggcggcggcgggtctggtggtggcggtggcagtggcggaggtggcggttcagcggaagccggtattaccgggacctggtccaatcaactcggctccacgtttatcgtgacagcaggcgcggatggcgcgctgacagggacgtacgagtccgcggtaggcaatgcggaaagccgctatgtgttgaccggtcgttacgattcggctccggctacggatggttccggtacagccttagggtggaccgttgcgtggaagaacaactcgaagaatgcccacagtgctaccacttggtcaggccagtatgttggcggggcggatgcgaaaatcaacactcagtggcttctgaccagcggaaccacgaatgccaatgcgtggaaatccacgctggtcggtcatgacacctttaccaaagtcaaaccgagtgcagcatcgcatcatcaccaccatcattaa

SEQ ID NO: 5 - DNA, 29 bp, synthetic construct
  misc_feature 1..29: note = Description of Artificial Sequence: Synthesized DNA
  source 1..29: mol_type = other DNA
catggtatatctccttcttaaagttaaac

SEQ ID NO: 6 - DNA, 30 bp, synthetic construct
  misc_feature 1..30: note = Description of Artificial Sequence: Synthesized DNA
  source 1..30: mol_type = other DNA
cgcagcttaattaacctaggctgctgccac

SEQ ID NO: 7 - DNA, 39 bp, synthetic construct
  misc_feature 1..39: note = Description of Artificial Sequence: Synthesized DNA
  source 1..39: mol_type = other DNA
aggagatataccatggtggacaacaaattcaacaaagag

SEQ ID NO: 8 - DNA, 41 bp, synthetic construct
  misc_feature 1..41: note = Description of Artificial Sequence: Synthesized DNA
  source 1..41: mol_type = other DNA
gttaattaagctgcgttaatgatggtggtgatgatgcgatg

SEQ ID NO: 9 - protein, 200 aa, synthetic construct
  REGION 1..200: note = Description of Artificial Sequence: Recombinant protein
MVDNKFNKEMRNAYWEIALLPNLNNQQKRAFIRSIYDDPSQSANLLAEAKKLNDAQAPKSGGGGGSGGGGGSGGGGGSAEAGITGTWSNQLGSTFIVTAGADGALTGTYESAVGNAESRYVLTGRYDSAPATDGSGTALGWTVAWKNNSKNAHSATTWSGQYVGGADAKINTQWLLTSGTTNANAWKSTLVGHDTFTKVK

SEQ ID NO: 10 - DNA, 600 bp, synthetic construct
  misc_feature 1..600: note = Description of Artificial Sequence: Recombinant DNA
  source 1..600: mol_type = other DNA
atggtggacaacaaattcaacaaagagatgcgcaatgcgtactgggaaattgccctgttaccgaacctgaacaaccagcagaaacgtgccttcattcgcagcatctatgacgatccaagccaatctgcgaatctgcttgcagaagcgaagaaactgaatgatgctcaagctccgaaaagcggaggcggcggcgggtctggtggtggcggtggcagtggcggaggtggcggttcagcggaagccggtattaccgggacctggtccaatcaactcggctccacgtttatcgtgacagcaggcgcggatggcgcgctgacagggacgtacgagtccgcggtaggcaatgcggaaagccgctatgtgttgaccggtcgttacgattcggctccggctacggatggttccggtacagccttagggtggaccgttgcgtggaagaacaactcgaagaatgcccacagtgctaccacttggtcaggccagtatgttggcggggcggatgcgaaaatcaacactcagtggcttctgaccagcggaaccacgaatgccaatgcgtggaaatccacgctggtcggtcatgacacctttaccaaagtcaaa

SEQ ID NO: 11 - protein, 191 aa, synthetic construct
  REGION 1..191: note = Description of Artificial Sequence: Recombinant protein
MVDNKFNKEMRNAYWEIALLPNLNNQQKRAFIRSIYDDPSQSANLLAEAKKLNDAQAPKGGGGSAEAGITGTWSNQLGSTFIVTAGADGALTGTYESAVGNAESRYVLTGRYDSAPATDGSGTALGWTVAWKNNSKNAHSATTWSGQYVGGADAKINTQWLLTSGTTNANAWKSTLVGHDTFTKVKPSAAS

SEQ ID NO: 12 - protein, 196 aa, synthetic construct
  REGION 1..196: note = Description of Artificial Sequence: Recombinant protein
MVDNKFNKEMRNAYWEIALLPNLNNQQKRAFIRSIYDDPSQSANLLAEAKKLNDAQAPKGGGGSGGGGSAEAGITGTWSNQLGSTFIVTAGADGALTGTYESAVGNAESRYVLTGRYDSAPATDGSGTALGWTVAWKNNSKNAHSATTWSGQYVGGADAKINTQWLLTSGTTNANAWKSTLVGHDTFTKVKPSAAS

SEQ ID NO: 13 - protein, 201 aa, synthetic construct
  REGION 1..201: note = Description of Artificial Sequence: Recombinant protein
MVDNKFNKEMRNAYWEIALLPNLNNQQKRAFIRSIYDDPSQSANLLAEAKKLNDAQAPKGGGGSGGGGSGGGGSAEAGITGTWSNQLGSTFIVTAGADGALTGTYESAVGNAESRYVLTGRYDSAPATDGSGTALGWTVAWKNNSKNAHSATTWSGQYVGGADAKINTQWLLTSGTTNANAWKSTLVGHDTFTKVKPSAAS

SEQ ID NO: 14 - DNA, 576 bp, synthetic construct
  misc_feature 1..576: note = Description of Artificial Sequence: Recombinant DNA
  source 1..576: mol_type = other DNA
atggtggacaacaaattcaacaaagagatgcgcaatgcgtactgggaaattgccctgttaccgaacctgaacaaccagcagaaacgtgccttcattcgcagcatctatgacgatccaagccaatctgcgaatctgcttgcagaagcgaagaaactgaatgatgctcaagctccgaaaggaggcggagggtctgcggaagccggtattaccgggacctggtccaatcaactcggctccacgtttatcgtgacagcaggcgcggatggcgcgctgacagggacgtacgagtccgcggtaggcaatgcggaaagccgctatgtgttgaccggtcgttacgattcggctccggctacggatggttccggtacagccttagggtggaccgttgcgtggaagaacaactcgaagaatgcccacagtgctaccacttggtcaggccagtatgttggcggggcggatgcgaaaatcaacactcagtggcttctgaccagcggaaccacgaatgccaatgcgtggaaatccacgctggtcggtcatgacacctttaccaaagtcaaaccgagtgcagcatcgtaa

SEQ ID NO: 15 - DNA, 591 bp, synthetic construct
  misc_feature 1..591: note = Description of Artificial Sequence: Recombinant DNA
  source 1..591: mol_type = other DNA
atggtggacaacaaattcaacaaagagatgcgcaatgcgtactgggaaattgccctgttaccgaacctgaacaaccagcagaaacgtgccttcattcgcagcatctatgacgatccaagccaatctgcgaatctgcttgcagaagcgaagaaactgaatgatgctcaagctccgaaaggaggcggagggtctggaggtggcggttcagcggaagccggtattaccgggacctggtccaatcaactcggctccacgtttatcgtgacagcaggcgcggatggcgcgctgacagggacgtacgagtccgcggtaggcaatgcggaaagccgctatgtgttgaccggtcgttacgattcggctccggctacggatggttccggtacagccttagggtggaccgttgcgtggaagaacaactcgaagaatgcccacagtgctaccacttggtcaggccagtatgttggcggggcggatgcgaaaatcaacactcagtggcttctgaccagcggaaccacgaatgccaatgcgtggaaatccacgctggtcggtcatgacacctttaccaaagtcaaaccgagtgcagcatcgtaa

SEQ ID NO: 16 - DNA, 606 bp, synthetic construct
  misc_feature 1..606: note = Description of Artificial Sequence: Recombinant DNA
  source 1..606: mol_type = other DNA
atggtggacaacaaattcaacaaagagatgcgcaatgcgtactgggaaattgccctgttaccgaacctgaacaaccagcagaaacgtgccttcattcgcagcatctatgacgatccaagccaatctgcgaatctgcttgcagaagcgaagaaactgaatgatgctcaagctccgaaaggaggcggagggtctggaggtggcggttcaggtggcggtggcagtgcggaagccggtattaccgggacctggtccaatcaactcggctccacgtttatcgtgacagcaggcgcggatggcgcgctgacagggacgtacgagtccgcggtaggcaatgcggaaagccgctatgtgttgaccggtcgttacgattcggctccggctacggatggttccggtacagccttagggtggaccgttgcgtggaagaacaactcgaagaatgcccacagtgctaccacttggtcaggccagtatgttggcggggcggatgcgaaaatcaacactcagtggcttctgaccagcggaaccacgaatgccaatgcgtggaaatccacgctggtcggtcatgacacctttaccaaagtcaaaccgagtgcagcatcgtaa

SEQ ID NO: 17 - protein, 127 aa, Streptomyces avidinii
AEAGITGTWYNQLGSTFIVTAGADGALTGTYESAVGNAESRYVLTGRYDSAPATDGSGTALGWTVAWKNNYRNAHSATTWSGQYVGGAEARINTQWLLTSGTTEANAWKSTLVGHDTFTKVKPSAAS

SEQ ID NO: 18 - protein, 58 aa, synthetic construct [sequence omitted]